European Patent Application EP 4 357 367 A1, published April 24, 2024. Title: 药物组合及用途. Applicant: 中山康方生物医药有限公司. The sequence listing filed with the application follows.

SEQUENCE LISTING (63 sequences)

SEQ ID NO: 1 - DNA, 372 bp, synthetic construct
  source 1..372: mol_type = other DNA
caggtcaagctgcaggagtctggacctgagctggtgaagcctggagcttcaatgaagatatcctgcaaggcttctggttactcattcactggctacaccatgaactgggtgaagcagagccatggaaagaaccttgaatggattggacttattaatccttacaataatattactaactacaaccagaagttcatgggcaaggccacatttactgtagacaagtcatccagcacagcctacatggaactcctcagactgacatctgaagactctggagtctatttctgtgcaagactcgactataggtcttattggggccaagggactctggtcactgtctctgcagccaaaacgacacccccatctgtctat

SEQ ID NO: 2 - protein, 124 aa, synthetic construct
QVKLQESGPELVKPGASMKISCKASGYSFTGYTMNWVKQSHGKNLEWIGLINPYNNITNYNQKFMGKATFTVDKSSSTAYMELLRLTSEDSGVYFCARLDYRSYWGQGTLVTVSAAKTTPPSVY

SEQ ID NO: 3 - DNA, 378 bp, synthetic construct
  source 1..378: mol_type = other DNA
caggctgttgtgactcaggaatctgcactcaccacatcacctggtgaaacagtcacactcacttgtcgctcaagtactggggctgttacaactagtaactttgccaactgggtccaagaaaaaccagatcatttattcactagtctaataggtggtaccaacaaccgagctccaggtgttcctgccagattctcaggctccctgattggagacaaggctgccctcaccatcacaggggcacagactgaggatgaggcaatatatttctgtgctctatggtacagcaaccattgggtgttcggtggaggaaccaaactgactgtcctaggccagcccaagtcttcgccatcagtcaccctgtttcaagggcaattctgc

SEQ ID NO: 4 - protein, 126 aa, synthetic construct
QAVVTQESALTTSPGETVTLTCRSSTGAVTTSNFANWVQEKPDHLFTSLIGGTNNRAPGVPARFSGSLIGDKAALTITGAQTEDEAIYFCALWYSNHWVFGGGTKLTVLGQPKSSPSVTLFQGQFC

SEQ ID NO: 5 - DNA, 345 bp, synthetic construct
  source 1..345: mol_type = other DNA
caggtgcagctggtggagtctggggccgagctggtgaagcccggcgcctccatgaagatctcttgcaaggccagcggatacagtttcactggctataccatgaactgggtcaaacaggctccaggacagggactggagtggatcgggctgattaatccttacaacaacatcaccaactacaaccagaagttcatgggaaaagcaacctttacagtggacaagagcatttccacagcctacatggaactgagccggctgacttcagacgatagcggggtctatttttgtgcaaggctggattatcgctcttactgggggcagggaactctggtcactgtctccgct

SEQ ID NO: 6 - protein, 115 aa, synthetic construct
QVQLVESGAELVKPGASMKISCKASGYSFTGYTMNWVKQAPGQGLEWIGLINPYNNITNYNQKFMGKATFTVDKSISTAYMELSRLTSDDSGVYFCARLDYRSYWGQGTLVTVSA

SEQ ID NO: 7 - DNA, 327 bp, synthetic construct
  source 1..327: mol_type = other DNA
caggctgtcgtcactcaggaaccttcactgactgtgagcccaggaggaactgtcaccctgacatgcggaagctccaccggagcagtgaccacatccaacttcgccaattgggtccaggaaaagccaggccaggcatttcgatccctgatcggaggcacaaacaatcgggcttcttgggtgcccgcaagattctcaggaagcctgctggggggaaaagccgctctgaccattagtggcgctcagcctgaggacgaagccgagtacttctgcgctctgtggtatagcaaccactgggtgtttggcgggggaacaaagctgactgtgctg

SEQ ID NO: 8 - protein, 109 aa, synthetic construct
QAVVTQEPSLTVSPGGTVTLTCGSSTGAVTTSNFANWVQEKPGQAFRSLIGGTNNRASWVPARFSGSLLGGKAALTISGAQPEDEAEYFCALWYSNHWVFGGGTKLTVL

SEQ ID NO: 9 - DNA, 345 bp, synthetic construct
  source 1..345: mol_type = other DNA
caggtgcagctggtcgagtctggggccgaagtgaagaaacccggcgcctcagtgaaggtcagctgcaaggccagcgggtacagtttcactggatataccatgaactgggtccgacaggcccctggccaggggctggagtggatcggcctgattaacccttacaacaacatcactaactacgcacagaagttccaggggagagtgacctttacagtggacaccagcatttccacagcctacatggaactgtcccggctgagatctgacgatacaggcgtgtacttctgcgctaggctggattaccgcagctattggggacagggcacactggtgactgtcagcgca

SEQ ID NO: 10 - protein, 115 aa, synthetic construct
QVQLVESGAEVKKPGASVKVSCKASGYSFTGYTMNWVRQAPGQGLEWIGLINPYNNITNYAQKFQGRVTFTVDTSISTAYMELSRLRSDDTGVYFCARLDYRSYWGQGTLVTVSA

SEQ ID NO: 11 - DNA, 327 bp, synthetic construct
  source 1..327: mol_type = other DNA
caggctgtcgtcactcaggaaccttcactgaccgtgtctcctggcgggactgtcaccctgacatgcggcagctccacaggggccgtgaccacaagtaacttcccaaattgggtccagcagaagccaggacaggctccccggagtctgatcggaggcaccaacaacaaggccagctggacacccgcacggttcagcggcagcctgctgggcggcaaggccgctctgacaattagcggagcccagcctgaggacgaagccgagtactattgcgctctgtggtactccaaccactgggtgttcggcggcggcaccaagctgactgtgctg

SEQ ID NO: 12 - protein, 109 aa, synthetic construct
QAVVTQEPSLTVSPGGTVTLTCGSSTGAVTTSNFPNWVQQKPGQAPRSLIGGTNNKASWTPARFSGSLLGGKAALTISGAQPEDEAEYYCALWYSNHWVFGGGTKLTVL

SEQ ID NO: 13 - DNA, 354 bp, synthetic construct
  source 1..354: mol_type = other DNA
gaggtcaaactggtggagagcggcggcgggctggtgaagcccggcgggtcactgaaactgagctgcgccgcttccggcttcgcctttagctcctacgacatgtcatgggtgaggcagacccctgagaagcgcctggaatgggtcgctactatcagcggaggcgggcgatacacctactatcctgactctgtcaaagggagattcacaattagtcgggataacgccagaaatactctgtatctgcagatgtctagtctgcggtccgaggatacagctctgtactattgtgcaaaccggtacggcgaagcatggtttgcctattggggacagggcaccctggtgacagtctctgcc

SEQ ID NO: 14 - protein, 118 aa, synthetic construct
EVKLVESGGGLVKPGGSLKLSCAASGFAFSSYDMSWVRQTPEKRLEWVATISGGGRYTYYPDSVKGRFTISRDNARNTLYLQMSSLRSEDTALYYCANRYGEAWFAYWGQGTLVTVSA

SEQ ID NO: 15 - DNA, 321 bp, synthetic construct
  source 1..321: mol_type = other DNA
gacattaagatgacacagtccccttcctcaatgtacgctagcctgggcgagcgagtgaccttcacatgcaaagcatcccaggacatcaacacatacctgtcttggtttcagcagaagccaggcaaaagccccaagaccctgatctaccgggccaatagactggtggacggggtccccagcagattctccggatctggcagtgggcaggattactccctgaccatcagctccctggagtatgaagacatgggcatctactattgcctgcagtatgatgagttccctctgacctttggagcaggcacaaaactggaactgaag

SEQ ID NO: 16 - protein, 107 aa, synthetic construct
DIKMTQSPSSMYASLGERVTFTCKASQDINTYLSWFQQKPGKSPKTLIYRANRLVDGVPSRFSGSGSGQDYSLTISSLEYEDMGIYYCLQYDEFPLTFGAGTKLELK

SEQ ID NO: 17 - DNA, 354 bp, synthetic construct
  source 1..354: mol_type = other DNA
gaagtgcagctggtcgagtctgggggagggctggtgcagcccggcgggtcactgcgactgagctgcgcagcttccggattcgcctttagctcctacgacatgtcctgggtgcgacaggcaccaggaaagggactggattgggtcgctactatctcaggaggcgggagatacacctactatcctgacagcgtcaagggccggttcacaatctctagagataacagtaagaacaatctgtatctgcagatgaacagcctgagggctgaggacaccgcactgtactattgtgccaaccgctacggggaagcatggtttgcctattgggggcagggaaccctggtgacagtctctagt

SEQ ID NO: 18 - protein, 118 aa, synthetic construct
EVQLVESGGGLVQPGGSLRLSCAASGFAFSSYDMSWVRQAPGKGLDWVATISGGGRYTYYPDSVKGRFTISRDNSKNNLYLQMNSLRAEDTALYYCANRYGEAWFAYWGQGTLVTVSS

SEQ ID NO: 19 - DNA, 321 bp, synthetic construct
  source 1..321: mol_type = other DNA
gacattcagatgactcagagcccctcctccatgtccgcctctgtgggcgacagggtcaccttcacatgccgcgctagtcaggatatcaacacctacctgagctggtttcagcagaagccagggaaaagccccaagacactgatctaccgggctaatagactggtgtctggagtcccaagtcggttcagtggctcagggagcggacaggactacactctgaccatcagctccctgcagcctgaggacatggcaacctactattgcctgcagtatgatgagttcccactgacctttggcgccgggacaaaactggagctgaag

SEQ ID NO: 20 - protein, 107 aa, synthetic construct
DIQMTQSPSSMSASVGDRVTFTCRASQDINTYLSWFQQKPGKSPKTLIYRANRLVSGVPSRFSGSGSGQDYTLTISSLQPEDMATYYCLQYDEFPLTFGAGTKLELK

SEQ ID NO: 21 - DNA, 1344 bp, synthetic construct
  source 1..1344: mol_type = other DNA
gaagtgcagctggtcgagtctgggggagggctggtgcagcccggcgggtcactgcgactgagctgcgcagcttccggattcgcctttagctcctacgacatgtcctgggtgcgacaggcaccaggaaagggactggattgggtcgctactatctcaggaggcgggagatacacctactatcctgacagcgtcaagggccggttcacaatctctagagataacagtaagaacaatctgtatctgcagatgaacagcctgagggctgaggacaccgcactgtactattgtgccaaccgctacggggaagcatggtttgcctattgggggcagggaaccctggtgacagtctctagtgccagcaccaaaggacctagcgtgtttcctctcgccccctcctccaaaagcaccagcggaggaaccgctgctctcggatgtctggtgaaggactacttccctgaacccgtcaccgtgagctggaatagcggcgctctgacaagcggagtccatacattccctgctgtgctgcaaagcagcggactctattccctgtccagcgtcgtcacagtgcccagcagcagcctgggcacccagacctacatctgtaacgtcaaccacaagccctccaacaccaaggtggacaagaaagtggagcccaaatcctgcgacaagacacacacctgtcccccctgtcctgctcccgaactcctcggaggccctagcgtcttcctctttcctcccaaacccaaggacaccctcatgatcagcagaacccctgaagtcacctgtgtcgtcgtggatgtcagccatgaggaccccgaggtgaaattcaactggtatgtcgatggcgtcgaggtgcacaacgccaaaaccaagcccagggaggaacagtacaactccacctacagggtggtgtccgtgctgacagtcctccaccaggactggctgaacggcaaggagtacaagtgcaaggtgtccaacaaggctctccctgcccccattgagaagaccatcagcaaggccaaaggccaacccagggagccccaggtctatacactgcctccctccagggacgaactcaccaagaaccaggtgtccctgacctgcctggtcaagggcttttatcccagcgacatcgccgtcgagtgggagtccaacggacagcccgagaataactacaagaccacccctcctgtcctcgactccgacggctccttcttcctgtacagcaagctgaccgtggacaaaagcaggtggcagcagggaaacgtgttctcctgcagcgtgatgcacgaagccctccacaaccactacacccagaaaagcctgtccctgagccccggcaaa

SEQ ID NO: 22 - protein, 448 aa, synthetic construct
EVQLVESGGGLVQPGGSLRLSCAASGFAFSSYDMSWVRQAPGKGLDWVATISGGGRYTYYPDSVKGRFTISRDNSKNNLYLQMNSLRAEDTALYYCANRYGEAWFAYWGQGTLVTVSSASTKGPSVFPLAPSSKSTSGGTAALGCLVKDYFPEPVTVSWNSGALTSGVHTFPAVLQSSGLYSLSSVVTVPSSSLGTQTYICNVNHKPSNTKVDKKVEPKSCDKTHTCPPCPAPELLGGPSVFLFPPKPKDTLMISRTPEVTCVVVDVSHEDPEVKFNWYVDGVEVHNAKTKPREEQYNSTYRVVSVLTVLHQDWLNGKEYKCKVSNKALPAPIEKTISKAKGQPREPQVYTLPPSRDELTKNQVSLTCLVKGFYPSDIAVEWESNGQPENNYKTTPPVLDSDGSFFLYSKLTVDKSRWQQGNVFSCSVMHEALHNHYTQKSLSLSPGK

SEQ ID NO: 23 - DNA, 642 bp, synthetic construct
  source 1..642: mol_type = other DNA
gacattcagatgactcagagcccctcctccatgtccgcctctgtgggcgacagggtcaccttcacatgccgcgctagtcaggatatcaacacctacctgagctggtttcagcagaagccagggaaaagccccaagacactgatctaccgggctaatagactggtgtctggagtcccaagtcggttcagtggctcagggagcggacaggactacactctgaccatcagctccctgcagcctgaggacatggcaacctactattgcctgcagtatgatgagttcccactgacctttggcgccgggacaaaactggagctgaagcgaactgtggccgctccctccgtcttcatttttcccccttctgacgaacagctgaaatcaggcacagccagcgtggtctgtctgctgaacaatttctaccctagagaggcaaaagtgcagtggaaggtcgataacgccctgcagtccggcaacagccaggagagtgtgactgaacaggactcaaaagatagcacctattccctgtctagtacactgactctgtccaaggctgattacgagaagcacaaagtgtatgcatgcgaagtgacacatcagggactgtcaagccccgtgactaagtcttttaaccggggcgaatgt

SEQ ID NO: 24 - protein, 214 aa, synthetic construct
DIQMTQSPSSMSASVGDRVTFTCRASQDINTYLSWFQQKPGKSPKTLIYRANRLVSGVPSRFSGSGSGQDYTLTISSLQPEDMATYYCLQYDEFPLTFGAGTKLELKRTVAAPSVFIFPPSDEQLKSGTASVVCLLNNFYPREAKVQWKVDNALQSGNSQESVTEQDSKDSTYSLSSTLTLSKADYEKHKVYACEVTHQGLSSPVTKSFNRGEC

SEQ ID NO: 25 - protein, 15 aa, synthetic construct
GGGGSGGGGSGGGGS

SEQ ID NO: 26 - protein, 20 aa, synthetic construct
GGGGSGGGGSGGGGSGGGGS

SEQ ID NO: 27 - protein, 8 aa, synthetic construct
GFAFSSYD

SEQ ID NO: 28 - protein, 8 aa, synthetic construct
ISGGGRYT

SEQ ID NO: 29 - protein, 11 aa, synthetic construct
ANRYGEAWFAY

SEQ ID NO: 30 - protein, 6 aa, synthetic construct
QDINTY

SEQ ID NO: 31 - skipped

SEQ ID NO: 32 - protein, 9 aa, synthetic construct
LQYDEFPLT

SEQ ID NO: 33 - protein, 8 aa, synthetic construct
GYSFTGYT

SEQ ID NO: 34 - protein, 8 aa, synthetic construct
INPYNNIT

SEQ ID NO: 35 - protein, 8 aa, synthetic construct
ARLDYRSY

SEQ ID NO: 36 - protein, 9 aa, synthetic construct
TGAVTTSNF

SEQ ID NO: 37 - skipped

SEQ ID NO: 38 - protein, 9 aa, synthetic construct
ALWYSNHWV

SEQ ID NO: 39 - DNA, 1344 bp, synthetic construct
  source 1..1344: mol_type = other DNA
gaagtgcagctggtcgagtctgggggagggctggtgcagcccggcgggtcactgcgactgagctgcgcagcttccggattcgcctttagctcctacgacatgtcctgggtgcgacaggcaccaggaaagggactggattgggtcgctactatctcaggaggcgggagatacacctactatcctgacagcgtcaagggccggttcacaatctctagagataacagtaagaacaatctgtatctgcagatgaacagcctgagggctgaggacaccgcactgtactattgtgccaaccgctacggggaagcatggtttgcctattgggggcagggaaccctggtgacagtctctagtgccagcaccaaagggcccagcgtgtttcctctcgccccctcctccaaaagcaccagcggaggaaccgctgctctcggatgtctggtgaaggactacttccctgaacccgtcaccgtgagctggaatagcggcgctctgacaagcggagtccatacattccctgctgtgctgcaaagcagcggactctattccctgtccagcgtcgtcacagtgcccagcagcagcctgggcacccagacctacatctgtaacgtcaaccacaagccctccaacaccaaggtggacaagaaagtggagcccaaatcctgcgacaagacacacacctgtcccccctgtcctgctcccgaagctgctggagcccctagcgtcttcctctttcctcccaaacccaaggacaccctcatgatcagcagaacccctgaagtcacctgtgtcgtcgtggatgtcagccatgaggaccccgaggtgaaattcaactggtatgtcgatggcgtcgaggtgcacaacgccaaaaccaagcccagggaggaacagtacaactccacctacagggtggtgtccgtgctgacagtcctccaccaggactggctgaacggcaaggagtacaagtgcaaggtgtccaacaaggctctccctgcccccattgagaagaccatcagcaaggccaaaggccaacccagggagccccaggtctatacactgcctccctccagggacgaactcaccaagaaccaggtgtccctgacctgcctggtcaagggcttttatcccagcgacatcgccgtcgagtgggagtccaacggacagcccgagaataactacaagaccacccctcctgtcctcgactccgacggctccttcttcctgtacagcaagctgaccgtggacaaaagcaggtggcagcagggaaacgtgttctcctgcagcgtgatgcacgaagccctccacaaccactacacccagaaaagcctgtccctgagccccggcaaa

SEQ ID NO: 40 - protein, 448 aa, synthetic construct
EVQLVESGGGLVQPGGSLRLSCAASGFAFSSYDMSWVRQAPGKGLDWVATISGGGRYTYYPDSVKGRFTISRDNSKNNLYLQMNSLRAEDTALYYCANRYGEAWFAYWGQGTLVTVSSASTKGPSVFPLAPSSKSTSGGTAALGCLVKDYFPEPVTVSWNSGALTSGVHTFPAVLQSSGLYSLSSVVTVPSSSLGTQTYICNVNHKPSNTKVDKKVEPKSCDKTHTCPPCPAPEAAGAPSVFLFPPKPKDTLMISRTPEVTCVVVDVSHEDPEVKFNWYVDGVEVHNAKTKPREEQYNSTYRVVSVLTVLHQDWLNGKEYKCKVSNKALPAPIEKTISKAKGQPREPQVYTLPPSRDELTKNQVSLTCLVKGFYPSDIAVEWESNGQPENNYKTTPPVLDSDGSFFLYSKLTVDKSRWQQGNVFSCSVMHEALHNHYTQKSLSLSPGK

SEQ ID NO: 41 - protein, 115 aa, synthetic construct
QVQLVESGAELVKPGASMKISCKASGYSFTGYTMNWVKQAPGQCLEWIGLINPYNNITNYNQKFMGKATFTVDKSISTAYMELSRLTSDDSGVYFCARLDYRSYWGQGTLVTVSA

SEQ ID NO: 42 - protein, 110 aa, synthetic construct
QAVVTQEPSLTVSPGGTVTLTCGSSTGAVTTSNFANWVQEKPGQAFRSLIGGTNNRASWVPARFSGSLLGGKAALTISGAQPEDEAEYFCALWYSNHWVFGCGTKLTVLR

SEQ ID NO: 43 - protein, 115 aa, synthetic construct
QVQLVESGAEVKKPGASVKVSCKASGYSFTGYTMNWVRQAPGQCLEWIGLINPYNNITNYAQKFQGRVTFTVDTSISTAYMELSRLRSDDTGVYFCARLDYRSYWGQGTLVTVSA

SEQ ID NO: 44 - protein, 110 aa, synthetic construct
QAVVTQEPSLTVSPGGTVTLTCGSSTGAVTTSNFPNWVQQKPGQAPRSLIGGTNNKASWTPARFSGSLLGGKAALTISGAQPEDEAEYYCALWYSNHWVFGCGTKLTVLR

SEQ ID NO: 45 - protein, 123 aa, synthetic construct [sequence omitted]

SEQ ID NO: 46 - DNA, 369 bp, synthetic construct
  source 1..369: mol_type = other DNA
gaggtgcagctggtcgagtccgggggggggctggtgcagccaggcgggtctctgaggctgagttgcgccgcttcagggtacaccttcacaaactatggaatgaattgggtgcgccaggcaccaggaaagggactggagtgggtcggctggatcaacacttacaccggggaacctacctatgcagccgactttaagcggcggttcaccttcagcctggatacaagcaaatccactgcctacctgcagatgaacagcctgcgagctgaggacaccgcagtctactattgtgctaaatatccccactactatgggagcagccattggtattttgacgtgtgggggcaggggactctggtgacagtgagcagc

SEQ ID NO: 47 - protein, 107 aa, synthetic construct [sequence omitted]

SEQ ID NO: 48 - DNA, 321 bp, synthetic construct
  source 1..321: mol_type = other DNA
gatattcagatgactcagagcccctcctccctgtccgcctctgtgggcgacagggtcaccatcacatgcagtgcttcacaggatatttccaactacctgaattggtatcagcagaagccaggaaaagcacccaaggtgctgatctacttcactagctccctgcactcaggagtgccaagccggttcagcggatccggatctggaaccgactttactctgaccatttctagtctgcagcctgaggatttcgctacatactattgccagcagtattctaccgtgccatggacatttggccaggggactaaagtcgagatcaag

SEQ ID NO: 49 - protein, 108 aa, synthetic construct
DIQMTQSPSSMSASVGDRVTFTCRASQDINTYLSWFQQKPGKSPKTLIYRANRLVSGVPSRFSGSGSGQDYTLTISSLQPEDMATYYCLQYDEFPLTFGAGTKLELKR

SEQ ID NO: 50 - protein, 453 aa, synthetic construct
EVQLVESGGGLVQPGGSLRLSCAASGYTFTNYGMNWVRQAPGKGLEWVGWINTYTGEPTYAADFKRRFTFSLDTSKSTAYLQMNSLRAEDTAVYYCAKYPHYYGSSHWYFDVWGQGTLVTVSSASTKGPSVFPLAPSSKSTSGGTAALGCLVKDYFPEPVTVSWNSGALTSGVHTFPAVLQSSGLYSLSSVVTVPSSSLGTQTYICNVNHKPSNTKVDKKVEPKSCDKTHTCPPCPAPELLGGPSVFLFPPKPKDTLMISRTPEVTCVVVDVSHEDPEVKFNWYVDGVEVHNAKTKPREEQYNSTYRVVSVLTVLHQDWLNGKEYKCKVSNKALPAPIEKTISKAKGQPREPQVYTLPPSRDELTKNQVSLTCLVKGFYPSDIAVEWESNGQPENNYKTTPPVLDSDGSFFLYSKLTVDKSRWQQGNVFSCSVMHEALHNHYTQKSLSLSPGK

SEQ ID NO: 51 - DNA, 1359 bp, synthetic construct
  source 1..1359: mol_type = other DNA
gaggtgcagctggtcgagtccgggggggggctggtgcagccaggcgggtctctgaggctgagttgcgccgcttcagggtacaccttcacaaactatggaatgaattgggtgcgccaggcaccaggaaagggactggagtgggtcggctggatcaacacttacaccggggaacctacctatgcagccgactttaagcggcggttcaccttcagcctggatacaagcaaatccactgcctacctgcagatgaacagcctgcgagctgaggacaccgcagtctactattgtgctaaatatccccactactatgggagcagccattggtattttgacgtgtgggggcaggggactctggtgacagtgagcagcgcaagcaccaaagggcccagcgtgtttcctctcgccccctcctccaaaagcaccagcggaggaaccgctgctctcggatgtctggtgaaggactacttccctgaacccgtcaccgtgagctggaatagcggcgctctgacaagcggagtccatacattccctgctgtgctgcaaagcagcggactctattccctgtccagcgtcgtcacagtgcccagcagcagcctgggcacccagacctacatctgtaacgtcaaccacaagccctccaacaccaaggtggacaagaaagtggagcccaaatcctgcgacaagacacacacctgtcccccctgtcctgctcccgaactcctcggaggccctagcgtcttcctctttcctcccaaacccaaggacaccctcatgatcagcagaacccctgaagtcacctgtgtcgtcgtggatgtcagccatgaggaccccgaggtgaaattcaactggtatgtcgatggcgtcgaggtgcacaacgccaaaaccaagcccagggaggaacagtacaactccacctacagggtggtgtccgtgctgacagtcctccaccaggactggctgaacggcaaggagtacaagtgcaaggtgtccaacaaggctctccctgcccccattgagaagaccatcagcaaggccaaaggccaacccagggagccccaggtctatacactgcctccctccagggacgaactcaccaagaaccaggtgtccctgacctgcctggtcaagggcttttatcccagcgacatcgccgtcgagtgggagtccaacggacagcccgagaataactacaagaccacccctcctgtcctcgactccgacggctccttcttcctgtacagcaaactgaccgtcgataaatctaggtggcagcagggcaacgtgttctcttgttccgtgatgcatgaagcactgcacaaccattatacccagaagtctctgagcctgtcccccggcaag

SEQ ID NO: 52 - protein, 450 aa, synthetic construct
EVQLVESGGGLVQPGGSLRLSCAASGYTFTNYGMNWVRQAPGKGLEWVGWINTYTGEPTYAADFKRRFTFSLDTSKSTAYLQMNSLRAEDTAVYYCAKYPHYYGSSHWYFDVWGQGTLVTVSSASTKGPSVFPLAPCSRSTSESTAALGCLVKDYFPEPVTVSWNSGALTSGVHTFPAVLQSSGLYSLSSVVTVPSSSLGTKTYTCNVDHKPSNTKVDKRVESKYGPPCPPCPAPEFLGGPSVFLFPPKPKDTLMISRTPEVTCVVVDVSQEDPEVQFNWYVDGVEVHNAKTKPREEQFNSTYRVVSVLTVLHQDWLNGKEYKCKVSNKGLPSSIEKTISKAKGQPREPQVYTLPPSQEEMTKNQVSLTCLVKGFYPSDIAVEWESNGQPENNYKTTPPVLDSDGSFFLYSRLTVDKSRWQEGNVFSCSVMHEALHNHYTQKSLSLSLGK

SEQ ID NO: 53 - DNA, 1350 bp, synthetic construct
  source 1..1350: mol_type = other DNA
gaggtgcagctggtcgagtccgggggggggctggtgcagccaggcgggtctctgaggctgagttgcgccgcttcagggtacaccttcacaaactatggaatgaattgggtgcgccaggcaccaggaaagggactggagtgggtcggctggatcaacacttacaccggggaacctacctatgcagccgactttaagcggcggttcaccttcagcctggatacaagcaaatccactgcctacctgcagatgaacagcctgcgagctgaggacaccgcagtctactattgtgctaaatatccccactactatgggagcagccattggtattttgacgtgtgggggcaggggactctggtgacagtgagcagcgcaagcaccaaagggccctcggtcttccccctggcgccctgctccaggagcacctccgagagcacagccgccctgggctgcctggtcaaggactacttccccgaaccggtgacggtgtcgtggaactcaggcgccctgaccagcggcgtgcacaccttcccggctgtcctacagtcctcaggactctactccctcagcagcgtggtgaccgtgccctccagcagcttgggcacgaagacctacacctgcaacgtagatcacaagcccagcaacaccaaggtggacaagagagttgagtccaaatatggtcccccatgcccaccatgcccagcacctgagttcctggggggaccatcagtcttcctgttccccccaaaacccaaggacactctcatgatctcccggacccctgaggtcacgtgcgtggtggtggacgtgagccaggaagaccccgaggtccagttcaactggtacgtggatggcgtggaggtgcataatgccaagacaaagccgcgggaggagcagttcaacagcacgtaccgtgtggtcagcgtcctcaccgtcctgcaccaggactggctgaacggcaaggagtacaagtgcaaggtctccaacaaaggcctcccgtcctccatcgagaaaaccatctccaaagccaaagggcagccccgagagccacaggtgtacaccctgcccccatcccaggaggagatgaccaagaaccaggtcagcctgacctgcctggtcaaaggcttctaccccagcgacatcgccgtggagtgggagagcaatgggcagccggagaacaactacaagaccacgcctcccgtgctggactccgacggctccttcttcctctacagcaggctaaccgtggacaagagcaggtggcaggaggggaatgtcttctcatgctccgtgatgcatgaggctctgcacaaccactacacacagaagtctctgagcctgtccctcggcaag

SEQ ID NO: 54 - protein, 453 aa, synthetic construct
EVQLVESGGGLVQPGGSLRLSCAASGYTFTNYGMNWVRQAPGKGLEWVGWINTYTGEPTYAADFKRRFTFSLDTSKSTAYLQMNSLRAEDTAVYYCAKYPHYYGSSHWYFDVWGQGTLVTVSSASTKGPSVFPLAPSSKSTSGGTAALGCLVKDYFPEPVTVSWNSGALTSGVHTFPAVLQSSGLYSLSSVVTVPSSSLGTQTYICNVNHKPSNTKVDKKVEPKSCDKTHTCPPCPAPEAAGGPSVFLFPPKPKDTLMISRTPEVTCVVVDVSHEDPEVKFNWYVDGVEVHNAKTKPREEQYNSTYRVVSVLTVLHQDWLNGKEYKCKVSNKALPAPIEKTISKAKGQPREPQVYTLPPSRDELTKNQVSLTCLVKGFYPSDIAVEWESNGQPENNYKTTPPVLDSDGSFFLYSKLTVDKSRWQQGNVFSCSVMHEALHNHYTQKSLSLSPGK

SEQ ID NO: 55 - DNA, 1359 bp, synthetic construct
  source 1..1359: mol_type = other DNA
gaggtgcagctggtcgagtccgggggggggctggtgcagccaggcgggtctctgaggctgagttgcgccgcttcagggtacaccttcacaaactatggaatgaattgggtgcgccaggcaccaggaaagggactggagtgggtcggctggatcaacacttacaccggggaacctacctatgcagccgactttaagcggcggttcaccttcagcctggatacaagcaaatccactgcctacctgcagatgaacagcctgcgagctgaggacaccgcagtctactattgtgctaaatatccccactactatgggagcagccattggtattttgacgtgtgggggcaggggactctggtgacagtgagcagcgcaagcaccaaagggcccagcgtgtttcctctcgccccctcctccaaaagcaccagcggaggaaccgctgctctcggatgtctggtgaaggactacttccctgaacccgtcaccgtgagctggaatagcggcgctctgacaagcggagtccatacattccctgctgtgctgcaaagcagcggactctattccctgtccagcgtcgtcacagtgcccagcagcagcctgggcacccagacctacatctgtaacgtcaaccacaagccctccaacaccaaggtggacaagaaagtggagcccaaatcctgcgacaagacacacacctgtcccccctgtcctgctcccgaagctgctggaggccctagcgtcttcctctttcctcccaaacccaaggacaccctcatgatcagcagaacccctgaagtcacctgtgtcgtcgtggatgtcagccatgaggaccccgaggtgaaattcaactggtatgtcgatggcgtcgaggtgcacaacgccaaaaccaagcccagggaggaacagtacaactccacctacagggtggtgtccgtgctgacagtcctccaccaggactggctgaacggcaaggagtacaagtgcaaggtgtccaacaaggctctccctgcccccattgagaagaccatcagcaaggccaaaggccaacccagggagccccaggtctatacactgcctccctccagggacgaactcaccaagaaccaggtgtccctgacctgcctggtcaagggcttttatcccagcgacatcgccgtcgagtgggagtccaacggacagcccgagaataactacaagaccacccctcctgtcctcgactccgacggctccttcttcctgtacagcaaactgaccgtcgataaatctaggtggcagcagggcaacgtgttctcttgttccgtgatgcatgaagcactgcacaaccattatacccagaagtctctgagcctgtcccccggcaag

SEQ ID NO: 56 - protein, 214 aa, synthetic construct
DIQMTQSPSSLSASVGDRVTITCSASQDISNYLNWYQQKPGKAPKVLIYFTSSLHSGVPSRFSGSGSGTDFTLTISSLQPEDFATYYCQQYSTVPWTFGQGTKVEIKRTVAAPSVFIFPPSDEQLKSGTASVVCLLNNFYPREAKVQWKVDNALQSGNSQESVTEQDSKDSTYSLSSTLTLSKADYEKHKVYACEVTHQGLSSPVTKSFNRGEC

SEQ ID NO: 57 - DNA, 642 bp, synthetic construct
  source 1..642: mol_type = other DNA
gatattcagatgactcagagcccctcctccctgtccgcctctgtgggcgacagggtcaccatcacatgcagtgcttcacaggatatttccaactacctgaattggtatcagcagaagccaggaaaagcacccaaggtgctgatctacttcactagctccctgcactcaggagtgccaagccggttcagcggatccggatctggaaccgactttactctgaccatttctagtctgcagcctgaggatttcgctacatactattgccagcagtattctaccgtgccatggacatttggccaggggactaaagtcgagatcaagcggaccgtggccgctcccagtgtcttcatttttccccctagcgacgaacagctgaaatccgggacagcctctgtggtctgtctgctgaacaacttctaccctagagaggcaaaagtgcagtggaaggtcgataacgccctgcagagtggcaattcacaggagagcgtgacagaacaggactccaaagattctacttatagtctgtcaagcacactgactctgagcaaggctgactacgaaaagcataaagtgtatgcatgtgaggtcacccaccaggggctgagcagtccagtcaccaagtcattcaacagaggcgagtgc

SEQ ID NO: 58 - protein, 8 aa, synthetic construct
GYTFTNYG

SEQ ID NO: 59 - protein, 8 aa, synthetic construct
INTYTGEP

SEQ ID NO: 60 - protein, 16 aa, synthetic construct
AKYPHYYGSSHWYFDV

SEQ ID NO: 61 - protein, 6 aa, synthetic construct
QDISNY

SEQ ID NO: 62 - skipped

SEQ ID NO: 63 - protein, 9 aa, synthetic construct
QQYSTVPWT